European Patent Application EP 4 223 880 A1, published August 9, 2023. Title: Mutant of Corynebacterium glutamicum with enhanced L-citrulline productivity and method for preparing L-citrulline using the same. Applicant: DAESANG CORPORATION. The sequence listing filed with the application follows.

SEQUENCE LISTING (6 sequences)

SEQ ID NO: 1 - DNA, 1302 bp, Artificial Sequence
  NCgl2816
atgacaaccgcagtagatcaaaactcaccgcccaagcagcaactcaacaagcgcgtcctgctgggcagcttgagtggcagcgttatcgaatggttcgacttcctggtttacggaaccgtcgccgcgctggtcttcaacaagatgtacttccccagcggcaacgagttcctctccacaatcctggcgtacgcatccttctccctgaccttcttcttccgccccattggtggcgtcatcttcgcccacatcggcgaccgcattgggcgtaagaagaccctgttcatcaccttgatgctcatgggtggcggcaccgtcgccattggtttgctgcccgactacaacgccatcggcatttgggcaccaatccttctgatgttcctccgcattttgcagggcatcggaattggcggcgaatggggtggcgcactgctcctggcatacgaatacgctccaaagaagcagcgtgggctctacggcgcagttcctcaaatgggcatttccctgggcatgctgcttgcagctggcgtgatctctctgctcaccctcatgccggaagatcagttcctcacctggggctggcgcatcccattcgtcggatccatcctcctagtgttcatcggcctgttcatccgaaacggccttgatgaaacccccgagttcaagcgtatccgcgattccggccagcaggtaaagatgcctctgaaggaagttctgaccaagtactggccagccgttctggtctccatcggcgcaaaagctgccgagaccggccccttctacatcttcggcacctacatcgttgcttacgcaaccaacttcctgaacatccgcgacaacattgtccttctggcagttgcttgcgccgccctcgttgccaccatctggatgccactgttcggatccttctccgaccgcgtcaaccgtgcagtgctctacaggatctgtgcatccgcaaccatcgtgctgattgtcccttactacttggtcctcaacaccggcgaaatttgggcactgtttatcactaccgtgattggcttcggcatcctctggggtagcgtcaacgcaatcctcggaaccgtcatcgcagaaaacttcgcacctgaggtccgctacaccggcgctaccctgggttaccaagtcggagcagcactcttcggcggtaccgcacccattatcgcagcatggctgttcgaaatctccggcggacaatggtggccaatcgccgtctacgtcgctgcatgttgccttctctctgtgatcgcctcgttcttcatccaacgcgtcgcgcaccaagagaactaa

SEQ ID NO: 2 - protein, 433 aa, Artificial Sequence
  NCgl2816
MTTAVDQNSPPKQQLNKRVLLGSLSGSVIEWFDFLVYGTVAALVFNKMYFPSGNEFLSTILAYASFSLTFFFRPIGGVIFAHIGDRIGRKKTLFITLMLMGGGTVAIGLLPDYNAIGIWAPILLMFLRILQGIGIGGEWGGALLLAYEYAPKKQRGLYGAVPQMGISLGMLLAAGVISLLTLMPEDQFLTWGWRIPFVGSILLVFIGLFIRNGLDETPEFKRIRDSGQQVKMPLKEVLTKYWPAVLVSIGAKAAETGPFYIFGTYIVAYATNFLNIRDNIVLLAVACAALVATIWMPLFGSFSDRVNRAVLYRICASATIVLIVPYYLVLNTGEIWALFITTVIGFGILWGSVNAILGTVIAENFAPEVRYTGATLGYQVGAALFGGTAPIIAAWLFEISGGQWWPIAVYVAACCLLSVIASFFIQRVAHQEN

SEQ ID NO: 3 - DNA, 25 bp, Artificial Sequence
  primer 1
tgatttacgccaagctccttatccg

SEQ ID NO: 4 - DNA, 40 bp, Artificial Sequence
  primer 2
ggaggggttttacttagattggtgacctcttctctgaaac

SEQ ID NO: 5 - DNA, 40 bp, Artificial Sequence
  primer 3
gtttcagagaagaggtcaccaatctaagtaaaacccctcc

SEQ ID NO: 6 - DNA, 19 bp, Artificial Sequence
  primer 4
ccggggatcctctagcgac